European Patent Application EP 4 745 244 A1, published May 20, 2026. Title: 工程生物遏制系统及方法. Applicant: 深圳华大生命科学研究院. The sequence listing filed with the application follows.

SEQUENCE LISTING (20 sequences)

SEQ ID NO: 1 - DNA, 54 bp, synthetic construct
  source 1..54: mol_type = other DNA
gaatgctggtcgctatactgggatggacgcaaagaagtttaataatcatattac

SEQ ID NO: 2 - DNA, 31 bp
gttttttctccttgacgttaaagtatagagg

SEQ ID NO: 3 - DNA, 24 bp, synthetic construct
  source 1..24: mol_type = other DNA
gacatggaggcccagaataccctc

SEQ ID NO: 4 - DNA, 51 bp, synthetic construct
  source 1..51: mol_type = other DNA
aaacttctttgcgtccatcccagtatagcgaccagcattcacatacgattg

SEQ ID NO: 5 - DNA, 64 bp, synthetic construct
  source 1..64: mol_type = other DNA
ttttgtgttgctcatgtcatagcattcaactacagatgaagacatggaggcccagaataccctc

SEQ ID NO: 6 - DNA, 75 bp, synthetic construct
  source 1..75: mol_type = other DNA
tcagtagcatattgttacacgaaggacaaaacgaaagcattatagttttttctccttgacgttaaagtatagagg

SEQ ID NO: 7 - DNA, 74 bp, synthetic construct
  source 1..74: mol_type = other DNA
gacattaccctgcagcgatttaacgggcgtcttggagaaaagaagagaaagacatggaggcccagaataccctc

SEQ ID NO: 8 - DNA, 85 bp, synthetic construct
  source 1..85: mol_type = other DNA
gtgaatcgttcaccctcaccactcactaggacaacattagaagtcaccattatagttttttctccttgacgttaaagtatagagg

SEQ ID NO: 9 - DNA, 84 bp, synthetic construct
  source 1..84: mol_type = other DNA
gtaaattctcttgtttttttttcttgatttcacttcttttcatgttcctttggaataatcgacatggaggcccagaataccctc

SEQ ID NO: 10 - DNA, 95 bp, synthetic construct
  source 1..95: mol_type = other DNA
ttcagcgtagaagacaccgtcagcgactagctttcttttcttagagattaaagcgaccattatagttttttctccttgacgttaaagtatagagg

SEQ ID NO: 11 - protein, 758 aa, Saccharomyces sp.
MAVNPELAPFTLSRGIPSFDDQALSTIIQLQDCIQQAIQQLNYSTAEFLAELLYAECSILDKSSVYWSDAVYLYALSLFLNKSYHTAFQISKEFKEYHLGIAYIFGRCALQLSQGVNEAILTLLSIINVFSSNSSNTRINMVLNSNLVHIPDLATLNCLLGNLYMKLDHSKEGAFYHSEALAINPYLWESYEAICKMRATVDLKRVFFDIAGKKSNSHNNNAASSFPSTSLSHFEPRSQPSLYSKTNKNGNNNINNNVNTLFQSSNSPPSTSASSFSSIQHFSRSQQQQANTSIRTCQNKNTQTPKNPAINSKTSSALPNNISMNLVSPSSKQPTISSLAKVYNRNKLLTTPPSKLLNNDRNHQNNNNNNNNNNNNNNNNNNNNNNNNIINKTTFKTPRNLYSSTGRLTTSKKNPRSLIISNSILTSDYSITLPEIMYNFALILRSSSQYNSFKAIRLFESQIPSHIKDTMPWCLVQLGKLHFEIINYDMSLKYFNRLKDLQPARVKDMEIFSTLLWHLHDKVKSSNLANGLMDTMPNKPETWCCIGNLLSLQKDHDAAIKAFEKATQLDPNFAYAYTLQGHEHSSNDSSDSAKTCYRKALACDPQHYNAYYGLGTSAMKLGQYEEALLYFEKARSINPVNVVLICCCGGSLEKLGYKEKALQYYELACHLQPTSSLSKYKMGQLLYSMTRYNVALQTFEELVKLVPDDATAHYLLGQTYRIVGRKKDAIKELTVAMNLDPKGNQVIIDELQKCHMQE

SEQ ID NO: 12 - protein, 781 aa, Saccharomyces sp.
MGSFPLAEFPLRDIPVPYSYRVSGGIASSGSVTALVTAAGTHRNSSTAKTVETEDGEEDIDEYQRKRAAGSGESTPERSDFKRVKHDNHKTLHPVNLQNTGAASVDNDGLHNLTDISNDAEKLLMSVDDGSAAPSTLSVNMGVASHNVAAPTTVNAATITGSDVSNNVNSATINNPMEEGALPLSPTASSPGTTTPLAKTTKTINNNNNIADLIESKDSIISPEYLSDEIFTAINNNLPHAYFKNLLFRLVANMDRSELSDLGTLIKDNLKRDLITSLPFEISLKIFNYLQFEDIINSLGVSQNWNKIIRKSTSLWKKLLISENFVSPKGFNSLNLKLSQKYPKLSQQDRLRLSFLENIFILKNWYNPKFVPQRTTLRGHMTSVITCLQFEDNYVITGADDKMIRVYDSINKKFLLQLSGHDGGVWALKYAHGGILVSGSTDRTVRVWDIKKGCCTHVFKGHNSTVRCLDIVEYKNIKYIVTGSRDNTLHVWKLPKESSVPDHGEEHGYPLVFHTPEENPYFVGVLRGHMASVRTVSGHGNIVVSGSYDNTLIVWDVAQMKCLYILSGHTDRIYSTIYDHERKRCISASMDTTIRIWDLENIWNNGECSYATNSASPCAKILGAMYTLQGHTALVGLLRLSDKFLVSAAADGSIRGWDANDYSRKFSYHHTNLSAITTFYVSDNILVSGSENQFNIYNLRSGKLVHANILKDADQIWSVNFKGKTLVAAVEKDGQSFLEILDFSKASKINYVSNPVNSSSSSSSLESISTSLGLTRTTIIP

SEQ ID NO: 13 - DNA, 32 bp, synthetic construct
  source 1..32: mol_type = other DNA
ctgtgtgcttaaaatatagtgtcttttttggg

SEQ ID NO: 14 - DNA, 23 bp, synthetic construct
  source 1..23: mol_type = other DNA
cttctgtctcaactgtcttagcc

SEQ ID NO: 15 - DNA, 27 bp, synthetic construct
  source 1..27: mol_type = other DNA
ccactgagagctgttcgtagataaatc

SEQ ID NO: 16 - DNA, 32 bp, synthetic construct
  source 1..32: mol_type = other DNA
cccaaaaaagacactatattttaagcacacag

SEQ ID NO: 17 - DNA, 23 bp, synthetic construct
  source 1..23: mol_type = other DNA
ggatcaaagtgcaagcaaaggtg

SEQ ID NO: 18 - DNA, 29 bp, synthetic construct
  source 1..29: mol_type = other DNA
cttgatttatcgagaatggagcattcagc

SEQ ID NO: 19 - DNA, 23 bp, synthetic construct
  source 1..23: mol_type = other DNA
ctcgccaaaagccatcttcgtac

SEQ ID NO: 20 - DNA, 23 bp, synthetic construct
  source 1..23: mol_type = other DNA
cacctttgcttgcactttgatcc